European Patent Specification EP 3 110 449 B1, published June 28, 2023. Title: MEDICAL USE OF A DPP-4 INHIBITOR. Applicant: Boehringer Ingelheim International GmbH. The sequence listing filed with the application follows.

SEQUENCE LISTING (10 sequences)

SEQ ID NO: 1 - DNA, 18 bp, Artificial Sequence
  source 1..18: /organism="Artificial Sequence" /note="PCR-primer collagen I forward" /mol_type="unassigned DNA"
tgccgatgtcgctatcca

SEQ ID NO: 2 - DNA, 25 bp, Artificial Sequence
  source 1..25: /organism="Artificial Sequence" /note="PCR-primer collagen I reverse " /mol_type="unassigned DNA"
tcttgcagtgataggtgatgttctg

SEQ ID NO: 3 - DNA, 26 bp, Artificial Sequence
  source 1..26: /organism="Artificial Sequence" /note="PCR-primer alpha-myosin heavy chain (MHC) forward " /mol_type="unassigned DNA"
tgtgaaaagattaaccggagtttaag

SEQ ID NO: 4 - DNA, 20 bp, Artificial Sequence
  source 1..20: /organism="Artificial Sequence" /note="PCR-primer alpha-myosin heavy chain (MHC) reverse" /mol_type="unassigned DNA"
tctgacttgcggaggtatcg

SEQ ID NO: 5 - DNA, 20 bp, Artificial Sequence
  source 1..20: /organism="Artificial Sequence" /note="PCR-primer beta-MHC forward " /mol_type="unassigned DNA"
gtgccaagggcctgaatgag

SEQ ID NO: 6 - DNA, 19 bp, Artificial Sequence
  source 1..19: /organism="Artificial Sequence" /note="PCR-primer beta-MHC reverse" /mol_type="unassigned DNA"
gcaaaggctccaggtctga

SEQ ID NO: 7 - DNA, 20 bp, Artificial Sequence
  source 1..20: /organism="Artificial Sequence" /note="PCR-primer atrial natriuretic peptide (ANP) forward" /mol_type="unassigned DNA"
atgggctccttctccatcac

SEQ ID NO: 8 - DNA, 18 bp, Artificial Sequence
  source 1..18: /organism="Artificial Sequence" /note="PCR-primer atrial natriuretic peptide (ANP) reverse" /mol_type="unassigned DNA"
tcttcggtaccggaagct

SEQ ID NO: 9 - DNA, 20 bp, Artificial Sequence
  source 1..20: /organism="Artificial Sequence" /note="PCR-primer RPL13a forward" /mol_type="unassigned DNA"
gatgaacaccaacccgtctc

SEQ ID NO: 10 - DNA, 20 bp, Artificial Sequence
  source 1..20: /organism="Artificial Sequence" /note="PCR-primer RPL13a reverse" /mol_type="unassigned DNA"
caccatccgctttttcttgt